European Patent Application EP 4 800 114 A1, published September 2, 2026. Title: 一种用于体外转录mRNA的质粒载体、构建方法及其应用. Applicant: 康希诺（上海）生物研发有限公司. The sequence listing filed with the application follows.

SEQUENCE LISTING (9 sequences)

SEQ ID NO: 1 - DNA, 82 bp, synthetic construct
  source 1..82: mol_type = other DNA
aatcagccgcacagattttttaaaacgcgccacgggatttttaaaccggtatttaacggtgtatgaatcccgttttatcttc

SEQ ID NO: 2 - DNA, 286 bp, synthetic construct
  source 1..286: mol_type = other DNA
ttcctgcgcgtccttatatggggctggataagaccggggaacaggaaatttttgatgccatcagaaaacgcgtcagcgccgctctgaggcaataaacagaatcaggcataaaatcagccgcacagattttttaaaacgcgccacgggatttttaaaccggtatttaacggtgtatgaatcccgttttatcttcctttcactttctttctccagtactcaaatagcataaccccagattttcccgcacctcccgcaaactgactgctcacaaaccatgatgagcagc

SEQ ID NO: 3 - DNA, 398 bp, synthetic construct
  source 1..398: mol_type = other DNA
tcatcagtggggcggtacacccgatatggcaccccgcccggcaggcgttcctgcgcgtccttatatggggctggataagaccggggaacaggaaatttttgatgccatcagaaaacgcgtcagcgccgctctgaggcaataaacagaatcaggcataaaatcagccgcacagattttttaaaacgcgccacgggatttttaaaccggtatttaacggtgtatgaatcccgttttatcttcctttcactttctttctccagtactcaaatagcataaccccagattttcccgcacctcccgcaaactgactgctcacaaaccatgatgagcagcaggacatgaaaaaacacgcgattggcattgccgcactgaatgcgctgtccattgacgatgacggc

SEQ ID NO: 4 - DNA, 164 bp, synthetic construct
  source 1..164: mol_type = other DNA
agcaggccattatcgccggcatggcggccgacgcgctgggctacgtcttgctggcgttcgcgacgcgaggctggatggccttccccattatgattcttctcgcttccggcggcatcgggatgcccgcgttgcaggccatgctgtccaggcaggtagatgacgac

SEQ ID NO: 5 - DNA, 282 bp, synthetic construct
  source 1..282: mol_type = other DNA
ttcggaatcttgcacgccctcgctcaagccttcgtcactggtcccgccaccaaacgtttcggcgagaagcaggccattatcgccggcatggcggccgacgcgctgggctacgtcttgctggcgttcgcgacgcgaggctggatggccttccccattatgattcttctcgcttccggcggcatcgggatgcccgcgttgcaggccatgctgtccaggcaggtagatgacgaccatcagggacagcttcaaggatcgctcgcggctcttaccagcctaacttcg

SEQ ID NO: 6 - DNA, 74 bp, synthetic construct
  source 1..74: mol_type = other DNA
caccacatagcagacccgccataaaacgccctgagaagcccgtgacgggcttttcttgtattatgggtagtttc

SEQ ID NO: 7 - DNA, 177 bp, synthetic construct
  source 1..177: mol_type = other DNA
ttgtttaaggtatgcaaatgcattaccttacccccttcaggcgcgtgtcgtgattttctaacctgtatttaacgggctttaaaatctgcgtgaagcgcctttgtatttttcccctggaagccacttcctgaaatcccgcaaaacccgccctgaaaattcccggcctatgctgccgga

SEQ ID NO: 8 - DNA, 236 bp, synthetic construct
  source 1..236: mol_type = other DNA
taggctaaaatcgcaaatatcgccacagaatcacgctaagggcgtttgaaaatcaatttatatcattttacgtctcaaaaaatttaaacgtgcttaaacgcatttaaacggcatttaaacgctattctaatttaaacctttctctaattttccacccctgactttcagcgttttattttaggctgatatatcacaaatccgcccttccctccctttaccgcaaaatagcggttatg

SEQ ID NO: 9 - DNA, 214 bp, synthetic construct
  source 1..214: mol_type = other DNA
gttttctctcttcaggtgggtgatttatcattgccagcgaatgaggggctgtattacctttataaaggctttacagcctctgttttataaccgcctccggttcaccgcattgctttccctgtccttctcccctgatgttttctaaagcagattaaaatcgccgggcctgcatttctcacaaactgtctccgacaacataacgcgggacagcaaa